European Patent Application EP 4 442 322 A1, published October 9, 2024. Title: Liver-specific CAR for use against immunologic rejection. Applicant: Medizinische Hochschule Hannover. The sequence listing filed with the application follows.

SEQUENCE LISTING (39 sequences)

SEQ ID NO: 1 - protein, 22 aa, synthetic construct
MDFQVQIFSFLLISASVIMSRT

SEQ ID NO: 2 - protein, 21 aa, synthetic construct
MWWRLWWLLLLLLLLWPMVWA

SEQ ID NO: 3 - protein, 20 aa, synthetic construct
MWWRLWWLLLLLLLLWPMVW

SEQ ID NO: 4 - protein, 21 aa, synthetic construct
MDFQVQIFSFLLISASVIMSR

SEQ ID NO: 5 - protein, 226 aa, synthetic construct
VPRDGGCKPCICTVPEVSSVFIFPPKPKDVLTITLTPKVTCVVVDISKDDPEVQFSWFVDDVEVHTAQTQPREEQFNSTFRSVSELPIMHQDWLNGKEFKCRVNSAAFPAPIEKTISKTKGRPKAPQVCTIPPPKEQMAKDKVSLTCMITDFFPEDITVEWQWNGQPAENYKNTQPIMDTDGSYFVYSKLNVQKSNWEAGNTFTCSVLHEGLHNHHTEKSLSHSPG

SEQ ID NO: 6 - protein, 57 aa, synthetic construct
SSVVPVLQKVNSTTTKPVLRTPSPVHPTGTSQPQRPEDCRPRGSVKGTGLDFACDIY

SEQ ID NO: 7 - protein, 83 aa, synthetic construct
FVPVFLPAKPTTTPAPRPPTPAPTIASQPLSLRPEASRPAAGGAVHTRGLDFADIYIWAPLAGTCGVLLLSLVITLYCNHRQL

SEQ ID NO: 8 - protein, 234 aa, synthetic construct
PAEPKSPDKTHTCPPCPAPPVAGPSVFLFPPKPKDTLMIARTPEVTCVVVDVSHEDPEVKFNWYVDGVEVHNAKTKPREEQYNSTYRVVSVLTVLHQDWLNGKEYKCKVSNKALPAPIEKTISKAKGQPREPQVYTLPPSRDELTKNQVSLTCLVKGFYPSDIAVEWESNGQPENNYKTTPPVLDSDGSFFLYSKLTVDKSRWQQGNVFSCSVMHEALHNHYTQKSLSLSPGKK

SEQ ID NO: 9 - protein, 25 aa, synthetic construct
VFLACVLGGSFGFLGFLGLCILCCV

SEQ ID NO: 10 - protein, 25 aa, synthetic construct
IWAPLAGICVALLLSLIITLICYHR

SEQ ID NO: 11 - protein, 42 aa, synthetic construct
NSRRNRLLQSDYMNMTPRRPGLTRKPYQPYAPARDFAAYRPL

SEQ ID NO: 12 - protein, 113 aa, synthetic construct
RAKFSRSAETAANLQDPNQLYNELNLGRREEYDVLEKKRARDPEMGGKQQRRRNPQEGVYNALQKDKMAEAYSEIGTKGERRRGKGHDGLYQGLSTATKDTYDALHMQTLAPR

SEQ ID NO: 13 - protein, 43 aa, synthetic construct
WTNSRRNRLLQSDYMNMTPRRPGLTRKPYQPYAPARDFAAYRP

SEQ ID NO: 14 - protein, 113 aa, synthetic construct; identical to SEQ ID NO: 12

SEQ ID NO: 15 - protein, 42 aa, synthetic construct
VRSKRSRLLHSDYMNMTPRRPGPTRKHYQPYAPPRDFAAYRS

SEQ ID NO: 16 - protein, 115 aa, synthetic construct
RVKFSRSADAPAYQQGQNQLYNELNLGRREEYDVLDKRRGRDPEMGGKPRRKNPQEGLYNELQKDKMAEAYSEIGMKGERRRGKGHDGLYQGLSTATKDTYDALHMQALPPRSSR

SEQ ID NO: 17 - protein, 72 aa, synthetic construct
DPKFWVLVVVGGVLACYSLLVTVAFIIFWVRSKRSRLLHSDYMNMTPRRPGPTRKHYQAYAAARDFAAYRSL

SEQ ID NO: 18 - protein, 112 aa, synthetic construct
RVKFSRSADAPAYQQGQNQLYNELNLGRREEYDVLDKRRGRDPEMGGKPRRKNPQEGLYNELQKDKMAEAYSEIGMKGERRRGKGHDGLYQGLSTATKDTYDALHMQALPPR

SEQ ID NO: 19 - protein, 19 aa, synthetic construct
ATNFSLLKQAGDVEENPGP

SEQ ID NO: 20 - protein, 429 aa, synthetic construct
MPNPRPAKPMAPSLALGPSPGVLPSWKTAPKGSELLGTRGSGGPFQGRDLRSGAHTSSSLNPLPPSQLQLPTVPLVMVAPSGARLGPSPHLQALLQDRPHFMHQLSTVDAHAQTPVLQVRPLDNPAMISLPPPSAATGVFSLKARPGLPPGINVASLEWVSREPALLCTFPRSGTPRKDSNLLAAPQGSYPLLANGVCKWPGCEKVFEEPEEFLKHCQADHLLDEKGKAQCLLQREVVQSLEQQLELEKEKLGAMQAHLAGKMALAKAPSVASMDKSSCCIVATSTQGSVLPAWSAPREAPDGGLFAVRRHLWGSHGNSSFPEFFHNMDYFKYHNMRPPFTYATLIRWAILEAPERQRTLNEIYHWFTRMFAYFRNHPATWKNAIRHNLSLHKCFVRVESEKGAVWTVDEFEFRKKRSQRPNKCSNPCP

SEQ ID NO: 21 - protein, 449 aa, synthetic construct
ATNFSLLKQAGDVEENPGPSMPNPRPAKPMAPSLALGPSPGVLPSWKTAPKGSELLGTRGSGGPFQGRDLRSGAHTSSSLNPLPPSQLQLPTVPLVMVAPSGARLGPSPHLQALLQDRPHFMHQLSTVDAHAQTPVLQVRPLDNPAMISLPPPSAATGVFSLKARPGLPPGINVASLEWVSREPALLCTFPRSGTPRKDSNLLAAPQGSYPLLANGVCKWPGCEKVFEEPEEFLKHCQADHLLDEKGKAQCLLQREVVQSLEQQLELEKEKLGAMQAHLAGKMALAKAPSVASMDKSSCCIVATSTQGSVLPAWSAPREAPDGGLFAVRRHLWGSHGNSSFPEFFHNMDYFKYHNMRPPFTYATLIRWAILEAPERQRTLNEIYHWFTRMFAYFRNHPATWKNAIRHNLSLHKCFVRVESEKGAVWTVDEFEFRKKRSQRPNKCSNPCP

SEQ ID NO: 22 - protein, 431 aa, synthetic construct
MPNPRPGKPSAPSLALGPSPGASPSWRAAPKASDLLGARGPGGTFQGRDLRGGAHASSSSLNPMPPSQLQLPTLPLVMVAPSGARLGPLPHLQALLQDRPHFMHQLSTVDAHARTPVLQVHPLESPAMISLTPPTTATGVFSLKARPGLPPGINVASLEWVSREPALLCTFPNPSAPRKDSTLSAVPQSSYPLLANGVCKWPGCEKVFEEPEDFLKHCQADHLLDEKGRAQCLLQREMVQSLEQQLVLEKEKLSAMQAHLAGKMALTKASSVASSDKGSCCIVAAGSQGPVVPAWSGPREAPDSLFAVRRHLWGSHGNSTFPEFLHNMDYFKFHNMRPPFTYATLIRWAILEAPEKQRTLNEIYHWFTRMFAFFRNHPATWKNAIRHNLSLHKCFVRVESEKGAVWTVDELEFRKKRSQRPSRCSNPTPGP

SEQ ID NO: 23 - protein, 259 aa, synthetic construct
MAQVQLVQSGAEVKKPGASVKVSCKASGYTFTSYYMHWVRQAPGQGPEWMGIINPSGGSTSYAQKFQGRVTMTRDTSTSTVYMELSSLRSEDTAVYYCARDAVGLRERYYYGMDVWGQGTTVTVSSGSASAPKLEEGEFSEARVDIVMTQSPSSLSASVGDRVTITCRASQSISSYLNWYQQKPGKAPKLLIYAASSLQSGVPSRFSGSGSGTDFTLTISSLQPEDFATYYCQQSYSTPFTFGGGTKVEIKRTVAAPSV

SEQ ID NO: 24 - protein, 309 aa, synthetic construct
MKYLLPTAAAGLLLLAAQPAMAQIQLVQSGGGLVQPGGSLRLSCAGSGYTFSDHYMDWVRQAPGKGLEWVGRIRYKANSYSTEYAASVKGRFTISRDDSRNSLFLQMNSLKTEDTAVYYCARIRDRYYFDYWGQGALVTVSSGSASAPKLEEGEFSEARVQSVLTQPPSVSGAPGQRVTISCTGSSSNVGAGYDVHWYQQLPGAAPKLLIYGNSNRPSGVPDRFSGSKSGTSASLAISGLQSEDEADYYCAAWDDSLNGVVFGGGTKLTVLGQPKAAPSVTLFPPSSAAAGSEQKLISEEDLSHHHHHH

SEQ ID NO: 25 - protein, 307 aa, synthetic construct
MKYLLPTAAAGLLLLAAQPAMAQVQLVQSGAEVKKPGASVKVSCKASGYTFTSYGISWVRQAPGQGLEWMGWISAYNGNTNYAQKLQGRVTMTTDTSTSTAYMELRSLRSDDTAVYYCARGYSYGDDFDYWGQGTLVTVSSGSASAPKLEEGEFSEARVNFMLTQPHSVSESPGKTVILSCTGTGGSIASNYVQWYQQRPGSAPTTVIYKDNERPSGVPDRFSGAIDSSSNSASLTISGLRTEDEADYYCQSYGSGNVVFGGGTKLTVLRQPKAAPSVTLFPPSSAAAGSEXKLISEEDLSHHHHHH

SEQ ID NO: 26 - protein, 292 aa, synthetic construct
MDFQVQIFSFLLISASVIMSRGVHSQVTLKESGGGLVQPGGSLRLSCAASGFTFSSYAMSWVRQAPGKGLEWVSAISGSGGSTYYADSVKGRFTISRDNSKNTLYLQMNSLRAEDTAVYYCAKDLKQWLEDYWGQGTLVTVSSGSASAPKLEEGEFSEARVDVVMTQSPSTLSASVGDRVTITCRASQSIGPWLAWYQQKPGEAPKLLLYKASILEGGVPSRFSGRGSGTEFTLTISSLQPDDFATYYCQQYNTFGPTFGQGTKLEIKRTVAAPSVFDPVPRDGGCKPCICT

SEQ ID NO: 27 - protein, 303 aa, synthetic construct
MDFQVQIFSFLLISASVIMSRGVHSQVQLVQSGAEVKKPGASVKVSCKASGYTFTGYYMHWVRQAPGQGLEWMGWINPNSGGTNYAQKFQGWVTMTRDTSISTAYMELSRLRSDDTAVYYCARKAVAADYFDYWGQGTLVTVSSGSASAPKLEEGEFSEARVNFMLTQPHSVSASPGKTVTISCTGSGGSIASHYVQWYQQRPGSAPTSVIYEDDQRPSGVPDRFSGSIDSSSNSASLTISGLKTEDEADYYCQSYDSSHQVFGGGTKLTVLGQPKASPSVTLFPPSSDPVPRDGGCKPCICT

SEQ ID NO: 28 - protein, 124 aa, synthetic construct
  REGION 1..25: note = FR1
  REGION 26..33: note = CDR1
  REGION 34..49: note = FR2
  REGION 50..58: note = CDR2
  REGION 59..96: note = FR3
  REGION 97..113: note = CDR3
  REGION 114..124: note = FR4
QVQLVQSGAEVKKPGASVKVSCKASGYTFTSYYMHWVRQAPGQGPEWMGIINPSGGSTSYAQKFQGRVTMTRDTSTSTVYMELSSLRSEDTAVYYCARDAVGLRERYYYGMDVWGQGTTVTVSS

SEQ ID NO: 29 - protein, 107 aa, synthetic construct
  REGION 1..26: note = FR1
  REGION 27..32: note = CDR1
  REGION 33..50: note = FR2
  REGION 51..53: note = CDR2
  REGION 54..88: note = FR3
  REGION 89..97: note = CDR3
  REGION 98..107: note = FR4
DIVMTQSPSSLSASVGDRVTITCRASQSISSYLNWYQQKPGKAPKLLIYAASSLQSGVPSRFSGSGSGTDFTLTISSLQPEDFATYYCQQSYSTPFTFGGGTKVEIK

SEQ ID NO: 30 - protein, 120 aa, synthetic construct
  REGION 1..25: note = FR1
  REGION 26..33: note = CDR1
  REGION 34..50: note = FR2
  REGION 51..60: note = CDR2
  REGION 61..98: note = FR3
  REGION 99..109: note = CDR3
  REGION 110..120: note = FR4
QIQLVQSGGGLVQPGGSLRLSCAGSGYTFSDHYMDWVRQAPGKGLEWVGRIRYKANSYSTEYAASVKGRFTISRDDSRNSLFLQMNSLKTEDTAVYYCARIRDRYYFDYWGQGALVTVSS

SEQ ID NO: 31 - protein, 111 aa, synthetic construct
  REGION 1..25: note = FR1
  REGION 26..34: note = CDR1
  REGION 35..51: note = FR2
  REGION 52..54: note = CDR2
  REGION 55..90: note = FR3
  REGION 91..101: note = CDR3
  REGION 102..111: note = FR4
QSVLTQPPSVSGAPGQRVTISCTGSSSNVGAGYDVHWYQQLPGAAPKLLIYGNSNRPSGVPDRFSGSKSGTSASLAISGLQSEDEADYYCAAWDDSLNGVVFGGGTKLTVL

SEQ ID NO: 32 - protein, 119 aa, synthetic construct
  REGION 1..25: note = FR1
  REGION 26..33: note = CDR1
  REGION 34..50: note = FR2
  REGION 51..58: note = CDR2
  REGION 59..96: note = FR3
  REGION 97..108: note = CDR3
  REGION 104..119: note = FR4
QVQLVQSGAEVKKPGASVKVSCKASGYTFTSYGISWVRQAPGQGLEWMGWISAYNGNTNYAQKLQGRVTMTTDTSTSTAYMELRSLRSDDTAVYYCARGYSYGDDFDYWGQGTLVTVSS

SEQ ID NO: 33 - protein, 110 aa, synthetic construct
  REGION 1..25: note = FR1
  REGION 26..33: note = CDR1
  REGION 34..50: note = FR2
  REGION 51..53: note = CDR2
  REGION 54..91: note = FR3
  REGION 92..100: note = CDR3
  REGION 101..110: note = FR4
NFMLTQPHSVSESPGKTVILSCTGTGGSIASNYVQWYQQRPGSAPTTVIYKDNERPSGVPDRFSGAIDSSSNSASLTISGLRTEDEADYYCQSYGSGNVVFGGGTKLTVL

SEQ ID NO: 34 - protein, 118 aa, synthetic construct
  REGION 1..25: note = FR1
  REGION 26..33: note = CDR1
  REGION 34..50: note = FR2
  REGION 51..58: note = CDR2
  REGION 59..96: note = FR3
  REGION 97..107: note = CDR3
  REGION 108..118: note = FR4
QVTLKESGGGLVQPGGSLRLSCAASGFTFSSYAMSWVRQAPGKGLEWVSAISGSGGSTYYADSVKGRFTISRDNSKNTLYLQMNSLRAEDTAVYYCAKDLKQWLEDYWGQGTLVTVSS

SEQ ID NO: 35 - protein, 107 aa, synthetic construct
  REGION 1..26: note = FR1
  REGION 27..32: note = CDR1
  REGION 33..49: note = FR2
  REGION 50..52: note = CDR2
  REGION 53..88: note = FR3
  REGION 89..97: note = CDR3
  REGION 98..107: note = FR4
DVVMTQSPSTLSASVGDRVTITCRASQSIGPWLAWYQQKPGEAPKLLLYKASILEGGVPSRFSGRGSGTEFTLTISSLQPDDFATYYCQQYNTFGPTFGQGTKLEIK

SEQ ID NO: 36 - protein, 119 aa, synthetic construct
  REGION 1..25: note = FR1
  REGION 26..33: note = CDR1
  REGION 34..50: note = FR2
  REGION 51..58: note = CDR2
  REGION 59..96: note = FR3
  REGION 97..108: note = CDR3
  REGION 109..119: note = FR4
QVQLVQSGAEVKKPGASVKVSCKASGYTFTGYYMHWVRQAPGQGLEWMGWINPNSGGTNYAQKFQGWVTMTRDTSISTAYMELSRLRSDDTAVYYCARKAVAADYFDYWGQGTLVTVSS

SEQ ID NO: 37 - protein, 110 aa, synthetic construct
  REGION 1..25: note = FR1
  REGION 26..33: note = CDR1
  REGION 34..50: note = FR2
  REGION 51..53: note = CDR2
  REGION 54..91: note = FR3
  REGION 92..100: note = CDR3
  REGION 101..110: note = FR4
NFMLTQPHSVSASPGKTVTISCTGSGGSIASHYVQWYQQRPGSAPTSVIYEDDQRPSGVPDRFSGSIDSSSNSASLTISGLKTEDEADYYCQSYDSSHQVFGGGTKLTVL

SEQ ID NO: 38 - DNA, 843 bp, synthetic construct
  source 1..843: mol_type = other DNA
  CDS 1..843: note = LNGFR; protein_id = 39; translation = MGAGATGRAMDGPRLLLLLLLGVSLGGAKEACPTGLYTHSGECCKACNLGEGVAQPCGANQTVCEPCLDSVTFSDVVSATEPCKPCTECVGLQSMSAPCVEADDAVCRCAYGYYQDETTGRCEACRVCEAGSGLVFSCQDKQNTVCEECPDGTYSDEANHVDPCLPCTVCEDTERQLRECTRWADAECEEIPGRWITRSTPPEGSDSTAPSTQEPEAPPEQDLIASTVAGVVTTVMGSSQPVVTRGTTDNLIPVYCSILAAVVVGLVAYIAFKRWNRGIL
atgggcgctggcgccacaggcagagctatggatggacctagactgctcctcctgctgctcctgggagtttctctcggcggagccaaagaggcctgtcctaccggactgtacacacactctggcgagtgctgcaaggcctgcaatctcggagaaggcgtggcacaaccttgcggcgctaatcagaccgtgtgcgagccttgtctggactccgtgacctttagcgacgtggtgtctgccaccgagccttgcaagccttgtaccgagtgtgtgggcctgcagagcatgtctgccccttgtgtggaagccgacgatgccgtgtgtagatgcgcctacggctactaccaggacgagacaacaggcagatgcgaggcctgtagagtgtgcgaagctggctctggactggtgttcagctgccaagacaagcagaacaccgtgtgtgaagagtgccccgacggcacctatagcgacgaagccaatcacgtggacccctgcctgccttgtactgtgtgcgaggacaccgagcggcagctgagagaatgtactagatgggccgacgccgagtgcgaagagatccctggaagatggatcaccagaagcaccccacctgagggcagcgattctacagccccaagcacacaagagcccgaggctcctccagaacaggacctgattgcctctacagtggccggcgtcgtgacaacagtgatgggatcttctcagcccgtggtcaccaggggcaccaccgataatctgatccccgtgtactgcagcatcctggccgctgtggttgtgggactcgtggcctatatcgccttcaagcggtggaaccggggcatcctctaa

SEQ ID NO: 39 - protein, 280 aa, synthetic construct
MGAGATGRAMDGPRLLLLLLLGVSLGGAKEACPTGLYTHSGECCKACNLGEGVAQPCGANQTVCEPCLDSVTFSDVVSATEPCKPCTECVGLQSMSAPCVEADDAVCRCAYGYYQDETTGRCEACRVCEAGSGLVFSCQDKQNTVCEECPDGTYSDEANHVDPCLPCTVCEDTERQLRECTRWADAECEEIPGRWITRSTPPEGSDSTAPSTQEPEAPPEQDLIASTVAGVVTTVMGSSQPVVTRGTTDNLIPVYCSILAAVVVGLVAYIAFKRWNRGIL